European Patent Application EP 4 763 197 A1, published June 24, 2026. Title: Functionalized ATP-hydrolyzing enzyme compositions. Applicant: MV BioTherapeutics SA. The sequence listing filed with the application follows.

SEQUENCE LISTING (2 sequences)

SEQ ID NO: 1 - protein, 254 aa, synthetic construct
MKTKNFLLFCIATNMIFIPSANALKAEGFLTQQTSPDSLSILPPPPAEDSVVFLADKAHYEFGRSLRDANRVRLASEDAYYENFGLAFSDAYGMDISRENTPILYQLLTQVLQDSHDYAVRNAKEYYKRVRPFVIYKDATCTPDKDEKMAITGSYPSGHASFGWAVALILAEINPQRKAEILRRGYEFGESRVICGAHWQSDVEAGRLMGASVVAVLHNTPEFTKSLSEAKKEFEELNTPTNELTPLEHHHHHH

SEQ ID NO: 2 - protein, 248 aa, Shigella flexneri
MKTKNFLLFCIATNMIFIPSANALKAEGFLTQQTSPDSLSILPPPPAEDSVVFLADKAHYEFGRSLRDANRVRLASEDAYYENFGLAFSDAYGMDISRENTPILYQLLTQVLQDSHDYAVRNAKEYYKRVRPFVIYKDATCTPDKDEKMAITGSYPSGHASFGWAVALILAEINPQRKAEILRRGYEFGESRVICGAHWQSDVEAGRLMGASVVAVLHNTPEFTKSLSEAKKEFEELNTPTNELTPLE